European Patent Specification EP 4 067 496 B1, published March 29, 2023. Title: ADAM6 MICE. Applicant: Regeneron Pharmaceuticals, Inc. The sequence listing filed with the application follows.

SEQUENCE LISTING (58 sequences)

SEQ ID NO: 1 - protein, 754 aa, Mus musculus
MLSLTWGMRLVERPVVPRVLLLLFALWLLLLVPVWCSQGHPTWRYISSEVVIPRKEIYHTKGLQAQRLLSYSLRFRGQRHIIHLRRKTLIWPRHLLLTTQDDQGALQMEYPFFPVDCYYIGYLEGILQSMVTVDTCYGGLSGVIKLDNLTYEIKPLNDSQSFEHLVSQIVSESDDTGPMNAWKHWSHNTGSPSSRLEYADGAPRLSSKNYATHPAAIKGHFQATHSVYSASGGDKLSSTVEYLFKVISLMDTYLTNLHMRYYVFLMTVYTEADPFSQDFRVPGGQAHTFYERVFYAHFRPDAGAIINKNSPGDDAVNPAERSICSPSALICLGQHGRNPLFLSIIITNRVGRSLGLKHDEGYCICQRRNTCIMFKNPQLTDAFSNCSLAEISNILNTPDLMPCLFYDRHVYYNTSLTYKFCGNFKVDNNEQCDCGSQKACYSDPCCGNDCRLTPGSICDKELCCANCTYSPSGTLCRPIQNICDLPEYCSGSKFICPDDTYLQDGTPCSEEGYCYKGNCTDRNIQCMEIFGVSAKNANIKCYDINKQRFRFGHCTRAEESLTFNACADQDKLCGRLQCTNVTNLPFLQEHVSFHQSVISGVTCFGLDEHRGTETADAGLVRHGTPCSRGKFCDRGACNGSLSRLGYDCTPEKCNFRGVCNNRRNCHCHFGWSPPKCKEEGHSGSIDSGSPPVQRRIIKQNLEPVVYLRILFGRIYFLFVALLFGIATRVGVTKIFRFEDLQAALRSWQEQAKDK

SEQ ID NO: 2 - protein, 756 aa, Mus musculus
MLSLTWGMRLVERPVVPRVLLLLFALWLLLLVPVWCSQGHPTWRYISSEVVIPRKEIYHTKGLQAQRLLSYSLHFRGQRHIIHLRRKTLIWPRHLLLTTQDDQGALQMDYPFFPVDCYYIGYLEGIPQSMVTVDTCYGGLSGVMKLDDLTYEIKPLNDSQSFEHLVSQIVSESDDTGPMNAWKHWSHNTGSPSSRLEYADGAPRISSKNYATHPAAIKGHFQATNSVYNSAAGDKLSSTVGYLFQVISLMDTYLTNLHMRYYVFLMTVYTNSDPFRLEFAVPGGSAYNYYVSVFYNKFKPDAGVLLNKYGPQDNQVNPAERSICSSLALICIGKYDRNPLFLSPIITNRVGRSLGLKYDEGYCVCQRRNTCIMFRHPQLTDAFSNCSLAEISNILNTPGLMPCLFYDRHVYYNTSLTYKFCGNFKVDNDEQCDCGSQKACYSDPCCGNDCRLTPGSICDKELCCANCTYSPSGTLCRPIQNICDLPEYCNGTKYICPDDTYLQDGTPCSEDGYCYKGNCTDRNIQCMEIFGVSAKNANIKCYDINKQRFRFGHCTRAEESLTFNACADQDKLCGRLQCTNVTNLPYLQEHVSFHQSIISGFTCFGLDEHRGTETTDAGMVRHGTPCSKSKFCDQGACSGSLSHLGYDCTPEKCSFRGVCNNHRNCHCHFGWKPPECKEEGLSGSIDSGSPPVQRHTIKQKQEPVVYLRILFGRIYFLFVALLFGIATRVGVTKIFRFEDLQATLRSGQGPARDKPK

SEQ ID NO: 3 - DNA, 13894 bp, Artificial Sequence
  synthetic
gtcctaaggtagcgagggatgacagattctctgttcagtgcactcagggtctgcctccacgagaatcaccatgccctttctcaagactgtgttctgtgcagtgccctgtcagtggaaatctggagagcatgcttccatgagcttgtgagtagtatatctagtaagccatggctttgtgttaatggtgatgttctacataccagttctctggcttaataatgaggtgatgattctatgttcctgtaacgcttcctcaactgggtcctaagtctttcttcactccatctattcctctaaggaatgatcctgaaaatcccatcacaaactataggagatgggaaccatcaaaaaacacagtgacaaagaggtgggaacgcatcagggttcaggaaccatattttaaaaagatatcgtaaataacttcttaaaagagatatagacaaatctccattaatacggagaccagaggcctaaggctaagaaccaatggtggctcaaggtctcctgctacccgaggagcaaacgtagagcagtttctaatgatttatttaaaatatagaatcaaaagtaccagtttgcaattttgaaagatttatttcagcaatgcaacaacatcaggtggtgccgagtccaacacgtcttatgtcccatgatataaacaaaggccatccagaactgtggactggagttctaccttgtcccctaatgacattcagattttttttccattctctttatcttagaggagacagggggctaactcattttacttgtcctttgcttgttcttgccaagaacgtaaagcagcttgcaagtcttcaaacctaaatatcttagtaactcctacacgagtggcaatgccaaagagcagtgcaacaaagaggaagtaaatacgaccaaagagtattcttaaatacactactggctctaggttctgttttattatgcgcctttgaaccggaggggacccactgtctatgctcccactgtgtccctcttctttgcactttggagggctccaaccaaaatggcaatggcaattccgacgattgttacacactcctctgaaattgcatttttctggggtgcagtcataacccaaacgagataaacttccattgcaagctcctcgatcacagaacttaccccttgaacacggggtaccatgtctcaccaatccagcatctgctgtttctgtcccacgatgttcatcaagcccaaagcaggtaaccccagagataaccgattgatggaatgaaacatgttcttgcaaaaatggaagattggtgacattggtacactgcaaccttccacacagcttgtcctgatcagcacaagcattgaatgtgaggctttcttctgctctagtacaatgcccaaatcgaaaccgttgtttgttgatgtcatagcacttaatattagcattcttagcacttacaccaaagatttccatgcattgtatgttgcgatcagtgcagttacctttatagcagtaaccctcttctgagcatggtgtcccatcttgcagataagtgtcatctgggcaaatgaacttagagccactacagtactctggaagatcacatatgttctggataggtctgcagagtgtcccagaaggactgtaagtgcaatttgcacagcataattctttatcacaaatgctaccaggtgttaacctgcaatcatttccacagcagggatctgaataacatgccttttgggagccacagtcacactgctcattgttatctactttgaagtttccacaaaacttataagtcaatgatgtattataataaacatgacggtcatagaaaagacatggcatcagatcaggagtattaagtatgttgcttatctctgcaagggaacaattgctgaaagcatctgttaattgaggatttttgaacatgatgcaggtgttccttctctggcagatacagtacccctcatcatgttttaggcctaaactccttccaacacgattggttattataatagataaaaataaaggatttcgaccatgttgaccaagacaaattagggctgagggagaacatatactcctctcagctggattaacagcatcatctcctggcgaattcttgttaattatagctcctgcatcaggcctaaaatgagcataaaatactctctcatagaaagtatgagcctgccctcctggaactcgaaaatcttgtgaaaatggatcagcctcggtatacacagtcatgagaaagacatagtaccgcatatgaagattggtcagataggtgtccattaaactaatgactttaaacaaatactcaacagtagatgaaagtttgtcacctccagaagcactatatacagaatgggttgcttgaaagtggccttttatagcagctggatgtgtagcgtaattcttactagatagtctgggagctccatctgcatattccaatctggaggagggagaacctgtattatggctccagtgcttccatgcattcataggccctgtgtcatcagactcagatactatctgagaaacaaggtgttcaaagctctgtgaatcattgaggggtttgatttcataggtaaggttatccaactttatgacccctgacaggcccccataacaagtatccacagtgaccatggattgcaggatcccctccaggtagccaatatagtaacaatctacaggaaaaaaggggtactccatctgtaaggctccttggtcatcttgagttgtcagcaacaagtgtctgggccaaatgagtgtctttctccgcaggtggatgatatgtctctggccccgaaaacgcaagctatacgagagcagtctttgtgcttgaagtcctttggtatggtagatctccttccgaggaataaccacctccgatgagatgtaacgccaagtgggatggccttgagaacaccagactggaaccaggaggagcagccagagtgcaaatagcaagaggaggaccctggggaccacaggtctttccactagcctcatgccccaggtcagagataacatcctgggtggagctaactccctctgctgtggccactgcctggtctagaaaatactgacagaggactaaaaacctcctcaggctcccaacctaagtggttacccagacaactggagttaggtaacagtcactgggtgtggcaggaattgagtctgaatgtgttagctgaggttgaggttaaatattgtcaaaagggatgtctataaatgtgcctggacaagaaaagtcagaagcagcaaggagtgtctctgacaggctcaatcctttcttttctttttttgaagttcaaaatatcatttccacgtgaatgtatttggttcccagtgtgactctgggtctctttctaggagtcaatatttctttatatcttggctcatgtttttcacagttgttctaacttcttgttttgttttgtttgtttgtttgtttgaaagttagaagtaaatactgtctatattagccttttagctataaatgattgtttttatttcttctaatcatgttttgtttgagttttggttaaactatttacaaatgagttttttttttccttttgggtgttgctcgaaagtttggagctttctgttaatattgtgttgttgtttctccaatattattagacctgagaattctacctgggtacctgtgaactccagaatttttaaaaattccatctcttgggaacattatctctgaccccgtctgaggccgaagtggctgtccccctccaacctttagtatctttctttcctgactattgggatttcttcaagcaatcaggctgatgggttctcagcagtgagaccagtagactgtcggtatgaacgtcgaagagtctgccacacactccgggttcatcaacagtgctttcgcgtctcttacttttgtagaaggaaatgcagcctctgagttttctccaagaaatcattgatgaaagggtgaaaagatgggtatcacccggagttcatgacaagccctggctcagacacgtgagcaaggtctacagccccaaagataggctgccctgcaacatgtatttataagataggagaaaaaaatgggtagttggagggttgatcaacttacttcctctcaaacatatatatctcatctaagtgtgcaggggaaaactctgtagaactactgggatacctgctcacccccaggagcctcatgaataagtctctgcttctgccttgtagccatgagcattactgcacctgatacccctgcagcttcctagggaagagggaggaagtgacttggcccctgtctggttaaggtaagaggagataaatcccttctcattgattagggtgagaggggtcatgtgctctatcattggtgacccagttgggacatgggtttataccaaagtcatcactctgaggttctgtgtaccaccaggctgaactcccatatcctacatggacataggacaacaccaagcagaaggaggttttaggactaaactgaaggacagagatgcggtttctaaacaactagggagtgccagggccagcctctctaaccactataggacactgtggagtctggttacaaagagagattactcaaggtccttagcactgattacagagcatatctcagatgccttctgctgaccagatgtatctttgcataatctgcctatccagattcagaaaattgatgccacatagccaagtggactttcaggaacagacgatttaaaaacaggcagagagatgtgagagaaaggagaaggagagagagaagggagagggagagaagagagagggagacggagaaggaaagagggagaaggagaaggagagaaggggcatggacagagggagggacagaaggagagaggagatagagagggggataaggaagaagggagggagggagagagagagaaggctaagtctttccatacctgggtcccaatacctcttataacccaagcacatggtttcacatatcacaatgcggttgggatatagataactgtaaatacttgtgaaaataatggggctgagatctggggttttcatgatagtttcaaagtcaccgtactgactaaaaccttccactggcccatctccagcttcctaatctgagggtatcaaatttcccactaagtgtgtttagaaagatctccacctttttgcccttgtcttccagtgccccacctacgttctggtctcccacatctgatgtcttctcagtgattctggccctgcctgctccacagctacaaaccccttcctataatgagctctgtgctgagccatcatcctgaatcaatccaccttaagcagatgttttgcttatttttcctgtgtccatactacagaggaaaggtaggcatgtagaagctgaagcatctcacctcattccaagcaccctcagtctctaaatgtgcccccttgtttccagaagtgcaacctcaagcatcttttattcattcatcttagagggccacatgtgctgtagtgttataagatgaaatttaaagcattaattattcctaacaagccaattaaacaagccaaaaacattcatcagtcattcccatggaacctctgaagcatcttcctgctctaaccttgggttttccagggctgctctgggatcacaggagctgtcctgtctaccagccatataaaggcagacctatcagaattacaccagacttctcaccatagactataaaagccagaatatcctggacagatgttatacagaaactaagagaacacaaatgccagcccaggctactatacccagcaaaactctcaattaccatcgatgaagaaaccaagatattccattacaagtccaaatttacacaatatctttccataaatccagccctacaaaggatagcagatggaaaactccaacacaggtaggaaaactacaccctagaaagagcactaaagtaatcatctttcaacacactcaaaagaagataaccacacaaacataattccacctctaacaacaaaaataaagtaggcaacaatcactattccttaatatctcttttaacatcaatggactcaattctccaataaaaagacatagactaacagactgaatacataaacaggacacagcattttgctgcataaagcaaacacagcgttacttttttttttctaaatgacattttttattagatattgtctttattgacatttcaaatgttatcccctttcctggtttaccctctgaaatcccctatctcctccccctccccctgctcaccaatccacccactcccacttccaggccctggcaatcccctatatttgggcatagagccttcacaggaccaaggtactctccttgcattgatgaccaactagtccattctctgctacaaatgcagctagatctatgagtcccaccatgttttcttttgttggtggtttcatgccagggagctcttggagtactgattggttcatattgttgttctccctatggggttacaaaacccttcaacttcttgggtcctttctctggctgcctcattggggaccttgtgcgaagtccaatggatgactgtgagcatccacttctgtatttgccaggcactggcagagcctctcagaagacagctatatcaagatcctggcagcaagctcttgttggtatccacaaaagtgtctggtggttgtctatgggatggatccccaaaggggcagtctctggatggtcattccttcagtctctgttccacactttgtctctttaactccttccatgactattttattcctccctctaagaaggaccgaagtattcatactttggtcttccttcttgaaattcatgtgttttgtgaattgtatctttgatattccgaacttctgggctaatatccacttatcagtgagtgaatatcatgtgtgttcttatgtgattgagttacctcactcaggatgatatcctccagaaccatccatttgtctaagaatttaatgaattcattgtttttaatagctgaggagtactccattgtgtaaatgtaccacattttctgtacccattgttctcttgagggacatctgggttctttaaagcttctggacattaaatataaggctgctatggaaatagtggagaatgtgtccttattacatgttggagcatcttctgggtatatgcccaggagtgctattgctggatcctctgatagtactatgtccaattttctgaggaactgccaaactgatttacagagtggttgtaccagcttgcaattccaccagcaatggagaaatgttccccttcctccacatcctcaccaacatctgctgtcacctcaatttgttcttagtgattcagacaggtgtgaggtggaatatcagggttgtttggcatttccctgatgactagtgatattgaaaaaaattttaagtgtttctcagccattcagtattcttcagttgagaattcactgtttagctctgtactcaggtttttttaatagggttatttggttttctggagtctaacgtcttgaattctttctatatattggatattagccctctgtcatatttaggattggtaaagatctttcccaatatgttggctgcctttttgtgtcctttgccttacagaacctttttaattttatgaggtcccatttgctaattcttcattttacagcacaagccattggtgttctgttcaaaaatctttccccctgaaccctatcttcgaggatcttccccactttctcctctataagtttcagtgtctctattattgtgctgaggggtaccgaagttcctattccgaagttcctattctctagaaagtataggaacttccctagggtttaaacccgcggtggagctctgatgtgggaacgcttcagtgttcaggaaccatatgatttatttaaaatatagaatcaaaagtaccaatttgcagttttgaaagatttattccagtgtaagcattagcaatgcaccaacatcaggtgatttctgaatccaacacgtcttatgtcctcatgatattaaaaaaaaaaaaaggccatccagaactgtgaacttgagttctaccttgttccctactgacattcagattttcttttttgcattctctttatcttacaggagacaggaggggagggctaactcattttactttggcttgtcccttgctggtccttgcccagaacgtaaagtagcttgcaagtcttcaaatctaaaaatcttagtaactcctacacgagtggcaatgccaaagagcagtgcaacaaagaggaagtaaatacgaccaaagagtattcttaaatacaccactggctcttgtttttgttttattgtgtgcctttgaactggaggggacccactgtctatgctcccacttagtccctcttctttgcactctggaggcttccaaccaaaatgacaatggcaattccgatgattgttacacactcctctaaaactgcatttttctggggtgcagtcataacccaaatgagataaacttccactgcaagctccttgatcacagaacttacttttggagcagggggtaccatgtctcaccattccagcatctgttgtttctgtcccacgatgttcatcaagcccaaagcaggtaaacccagagataatcgattgatggaatgaaacatgttcttgcaaatatggaagattggtgacattggtacactgcaaccttccacacagcttgtcctgatcagcacaagcattgaatgtgaggctttcttctgctctagtacaatgcccaaatcgaaaccgttgtttgttgatgtcatagcacttaatattagcattcttagcacttacaccaaagatttccatgcattgtatgttgcgatcagtgcagttacctttatagcagtaaccatcttctgagcatggtgtcccatcttgcagataagtgtcatctgggcaaatgtatttagtcccattacagtactctggaagatcacatatgttctggataggtctgcagagtgtcccagaaggactgtaagtgcaatttgcacagcataattctttatcacaaatgctaccaggtgttaacctgcaatcatttccacagcagggatctgaataacatgccttttgggagccacagtcacactgctcatcgttatctactttgaagtttccacaaaacttataagtcaatgatgtattataataaacatgacggtcatagaaaagacatggcatcagaccaggagtattaagtatgttgcttatctctgcaagggaacaattgctgaaagcatctgttaattgaggatgtctgaacataatgcaggtgttccttctctggcagacacagtacccctcatcatattttaagcctaaactccttccaacacgattggttattataggagataaaaataaaggatttcgatcatatttaccaatacaaattagggctaaggaagaacatatactcctctcagctggattaacctggttatcttgtggcccatacttattaagtaaaactcctgcatcaggcttaaatttattataaaagactgacacatagtaattataagccgaccctcctggaactgcaaactcaagtcgaaatggatcagaattggtgtacacagtcatgagaaagacatagtaccgcatatgaagattggtcagataggtgtccattaaactaatgacttgaaacaaatacccaacagtagatgaaagtttgtcacctgcagcagaattatatacagaattggttgcttgaaagtggccttttatagcagctggatgtgtagcgtagttcttactagatattctgggagctccatctgcatattccaatctggaggagggagaacctgtattatggctccagtgcttccatgcattcataggccctgtgtcatcagactcagatactatctgagaaacaaggtgttcaaagctctgtgaatcattgaggggtttgatttcataggtaaggtcatctaacttcatgacccctgacaggcccccataacaagtatccacagtgaccatggattgtgggatcccctccaggtagccaatatagtaacaatctacaggaaaaaaggggtaatccatctgtaaggctccttggtcatcttgagttgtcagcaacaagtgtctgggccaaatgagtgtctttctccgcaggtggatgatatgtctctggccccgaaaatgcaagctatatgagagcagtctttgtgcttgaagtcctttggtatggtagatctccttccgaggaataaccacctccgatgagatgtaacgccaagtaggatggccttgagaacaccagactggaaccaggaggagcagccagagtgcaaatagcaagaggaggaccctggggaccacaggtctttccactagcctcatgccccaggtcagagataacatcctgggtggagctaaatccctctgctgtggccactgcctggtctagaaaatactgacagaggactaaaaacctcctcaggctcccaacctaagtggttacccagacaactggagttaggtaacagtcactgggtgtggcaggaattgagtctgaatgtgttagctgaggttgaggttaaatattgtcaaaagggatgtctataaatgtgcctggacaagaaaagtcagaagcagcaaggagtgtctctgacaggctcaatcctttcttttctttttttgaagttcaaaatatcatttccacgtgaatgtatttggttcccagtgtgactctgggtctctttctaggagtcaatatttctttatatcttggctcatgtttctcacagttgttctaatttcttgttttgttttgtttgtttgtttgaacgttagtagtaaatactgtctatattagccttttagctataaatgattgtttttatttcttctaatcatattttgtttgagttttggttaaactatttacaaatgagttttttttttttccttttgggtgttgctcgaaagtttggagctttctgttaatattgtgttgttatttttccaatattattagacctgagaattctatctgggtacctgtgaactctagaatttttaaaaattccatctcttgggaacattacctctgaccccgtctgaggccgaagtggctgtccccctccaacctttagtatctttctttcctgactattgggatttcttcaagcaatcaggctgatgggttctcagcagtgagaccagtagactgccggtatgaacgtcgaagagactgccacacactccaggttcatcaacagtgctttcgcgtctcttacttttgtagaaggaaaagcagcctctgagttatctccaagaaatcattaatgaaagagttaaaagatgggtatcacccggagttcatgacaagccctggctcagacacgtgagcaaggtctacagccccaaagataggctgccctgcaacatgtatttataagatagaagaaaaaaatgggtggttggagggttgatcaacttacttcctctcaaacatatatatctcatctaagtgtgcaggggaaaactctgtaggactactgggattgttattatcattattattattattattattattattattattattattattattaacttaaggcattttattagatattttcttcatttagttttcaaatgttatccccggaacctcctatactctctccctgccctgctccccaacccacccactcctacatcctggccctggcattcccctatactgtggcagatgatcttcgtaagaccaagagcctttcctcccattgatggcctactaggctatcctcttttacatatgcaactagagtcacagctctggggaggtattgcttagttcatattgtttttcctcctatagggttgcagatccctttagctccttgggtactttctctagctcctccattgggggccctgtgttccatccaatagatgactgtgagcatccacttctgtatttgccaggtattggcatggatcttactgcaccttctgaactctctaagcagctttcctggtcacctccaggagcctcatgaataagtctctgcttcccccttgtggctatgagcattactgcacctgatacaccctgcagcttcctagggaagagggaggaagtggcttggcccctgtctggttaaggtaagaggagataaatcccttctcatgaattagggtgagaagggtcatgtgctctatcattggtgaccaacttggggacatgggcttatacagtcatcactctgaggctctgtgtaccaccagactgaactcccatatcctacatgcacataggacaacaccaagtagaaggaggttttaggactaaactgaaggacagagatggggtttctaaacaactagggagtgccagggccagcctctctaaccactataggacactatggagtctggttacaaagagagattactcaaggtccttagcactgattacagagcatatctcagatgccttctgctgaccagatgtatctttgcataatctgcctatccagattcagaaaattgatgccacatagccaagtggactttcaggaacagacgatttaaaaacaggcagagagatgtgagagaaaggagaaggagagagagaagggagagggagagaagagagagggagacggagaaggaaagagggagaaggagaaggagagaaggggcatggacagagggagggacagaaggagagaggagatagagagggggataaggaagaaaggagggagggagagagagagaaggctaagtctttccatacctgggtcccaatacctcttataacccaagcacatggtttcagatatcacaatgcggttgggatatagataactgtaaatacttgtgaaaataatggggctgagatctggggttttcatgatagtttcaaagtcactgtactgactaaaaccttccactggcccatctccagcttgttaatctgagggtatcaaatttcccactaagtgtgtttagaaagatctccacctttttgccctagtcttccagtgccccacctacgttctggtctcccacatctgatgtcttctcagtgattctggccctgcctgctccacagctacaaaccccttcctataatgagctctgtgctgagccatcatcctgaatcaatccaccttaagcagatgttttgcttatttttcctgtgtccatactacagaggaagggtaggcatgtagaagctgaggcatctcatctcactctaagcaccctcagtctctaaatgtgcccctttgtttccagcagttcagcctcaagcatcttttattcactcgtcttagagggacacatgtgctgtagtgttataagatgaaatttaaagcattagttattcccaacaagccaattaaacaagccaaaaacattcatcagtcattcccatggaacctctgaagcatcttcctgctctaaccttgagtttcctagggctgctgtgggatcacaggagctgtcctgtttaccagcctatcctgtcccacgggattcagttattagtgggtgcgagggggaccgcaaacctggaagaaaatgggattggaagagaaaagagaaacgaagaccaagtagatcttttcctatcaaggtcttcgtttattaggctgaggtgcctggtgtaaagcatgcatcgcggggaataggaaggggtcgagggggaattttacaaagaacaaagaagcgggcatctgctgacatgagggccgaagtcaggctccaggcagcgggagctccaccgcggtggcgccatttcattacctctttctccgcacccgacatagataaagctta

SEQ ID NO: 4 - DNA, 251 bp, Artificial Sequence
  synthetic
ccagcttcattagtaatcgttcatctgtggtaaaaaggcaggatttgaagcgatggaagatgggagtacggggcgttggaagacaaagtgccacacagcgcagccttcgtctagacccccgggctaactataacggtcctaaggtagcgaggggatgacagattctctgttcagtgcactcagggtctgcctccacgagaatcaccatgccctttctcaagactgtgttctgtgcagtgccctgtcagtgg

SEQ ID NO: 5 - DNA, 245 bp, Artificial Sequence
  synthetic
aggggtcgagggggaattttacaaagaacaaagaagcgggcatctgctgacatgagggccgaagtcaggctccaggcagcgggagctccaccgcggtggcgccatttcattacctctttctccgcacccgacatagataaagcttatcccccaccaagcaaatccccctacctggggccgagcttcccgtatgtgggaaaatgaatccctgaggtcgattgctgcatgcaatgaaattcaactag

SEQ ID NO: 6 - DNA, 21 bp, Artificial Sequence
  synthetic
caggtacagctgcagcagtca

SEQ ID NO: 7 - DNA, 21 bp, Artificial Sequence
  synthetic
ggagatggcacaggtgagtga

SEQ ID NO: 8 - DNA, 17 bp, Artificial Sequence
  synthetic
tccaggactggtgaagc

SEQ ID NO: 9 - DNA, 24 bp, Artificial Sequence
  synthetic
tagtcccagtgatgagaaagagat

SEQ ID NO: 10 - DNA, 24 bp, Artificial Sequence
  synthetic
gagaacacagaagtggatgagatc

SEQ ID NO: 11 - DNA, 17 bp, Artificial Sequence
  synthetic
tgagtccagtccaggga

SEQ ID NO: 12 - DNA, 28 bp, Artificial Sequence
  synthetic
aaaaattgagtgtgaatggataagagtg

SEQ ID NO: 13 - DNA, 21 bp, Artificial Sequence
  synthetic
aaccctggtcagaaactgcca

SEQ ID NO: 14 - DNA, 19 bp, Artificial Sequence
  synthetic
agagaaacagtggatacgt

SEQ ID NO: 15 - DNA, 22 bp, Artificial Sequence
  synthetic
aactacgcacagaagttccagg

SEQ ID NO: 16 - DNA, 18 bp, Artificial Sequence
  synthetic
gctcgtggatttgtccgc

SEQ ID NO: 17 - DNA, 16 bp, Artificial Sequence
  synthetic
cagagtcacgattacc

SEQ ID NO: 18 - DNA, 19 bp, Artificial Sequence
  synthetic
tgagcagcaccctcacgtt

SEQ ID NO: 19 - DNA, 23 bp, Artificial Sequence
  synthetic
gtggcctcacaggtatagctgtt

SEQ ID NO: 20 - DNA, 18 bp, Artificial Sequence
  synthetic
accaaggacgagtatgaa

SEQ ID NO: 21 - DNA, 33 bp, Artificial Sequence
  synthetic
gctagtagtggggcctacaggccttttgatatc

SEQ ID NO: 22 - DNA, 48 bp, Artificial Sequence
  synthetic
gcaaaagcccaggggagtgggagctactacacctatgcttttgatatc

SEQ ID NO: 23 - DNA, 42 bp, Artificial Sequence
  synthetic
gcgagagagggtatagtgggaactactgaggactttgattac

SEQ ID NO: 24 - DNA, 33 bp, Artificial Sequence
  synthetic
gcgagagggacagtgggagccctctttgactac

SEQ ID NO: 25 - DNA, 36 bp, Artificial Sequence
  synthetic
gcgaaacctagtgggagctactcctggttcgacccc

SEQ ID NO: 26 - DNA, 45 bp, Artificial Sequence
  synthetic
gcgagaggaggagggtataactggaactcgaatgcttttgatatc

SEQ ID NO: 27 - DNA, 33 bp, Artificial Sequence
  synthetic
gcgagaggatataactggaactactttgactac

SEQ ID NO: 28 - DNA, 39 bp, Artificial Sequence
  synthetic
gcgaaagagtataactggaaccactggtactttgactac

SEQ ID NO: 29 - DNA, 33 bp, Artificial Sequence
  synthetic
gcgagagagataactggaaccccctttgactac

SEQ ID NO: 30 - DNA, 39 bp, Artificial Sequence
  synthetic
gcgaggggatataactggaacttttctttttttgactac

SEQ ID NO: 31 - DNA, 36 bp, Artificial Sequence
  synthetic
gcgagaggtaactggaactctctgggctttgactac

SEQ ID NO: 32 - DNA, 39 bp, Artificial Sequence
  synthetic
gcgaaaagggctactatggttcggggagctcttgactac

SEQ ID NO: 33 - DNA, 60 bp, Artificial Sequence
  synthetic
gcgagagatattactatggttcggggagttattataacgaaggtctacggtatggacgtc

SEQ ID NO: 34 - DNA, 27 bp, Artificial Sequence
  synthetic
gcgagagagtatagcagctttgactac

SEQ ID NO: 35 - DNA, 33 bp, Artificial Sequence
  synthetic
gcgagagagagtatagcagctcgttgtgactac

SEQ ID NO: 36 - DNA, 42 bp, Artificial Sequence
  synthetic
gcaagagaggataggagctcgcccctcgggtactttgactac

SEQ ID NO: 37 - DNA, 24 bp, Artificial Sequence
  synthetic
gcgagagatcttggggaaggctac

SEQ ID NO: 38 - DNA, 30 bp, Artificial Sequence
  synthetic
accacccataactggggagggtttgactac

SEQ ID NO: 39 - DNA, 18 bp, Artificial Sequence
  synthetic
gcgagagataggggaccg

SEQ ID NO: 40 - DNA, 30 bp, Artificial Sequence
  synthetic
caacagagttatagtacccctccggagacg

SEQ ID NO: 41 - DNA, 27 bp, Artificial Sequence
  synthetic
caacagcttaatagttaccctcggacg

SEQ ID NO: 42 - DNA, 26 bp, Artificial Sequence
  synthetic
caacagcttaatagttaccattcact

SEQ ID NO: 43 - DNA, 27 bp, Artificial Sequence
  synthetic
caacattttaatagttacccgctcact

SEQ ID NO: 44 - DNA, 27 bp, Artificial Sequence
  synthetic
cagcagtataataactggcctctcact

SEQ ID NO: 45 - DNA, 27 bp, Artificial Sequence
  synthetic
ctacagcataatagttacccgtggacg

SEQ ID NO: 46 - DNA, 27 bp, Artificial Sequence
  synthetic
ctacagcataatagttaccctcggacg

SEQ ID NO: 47 - DNA, 27 bp, Artificial Sequence
  synthetic
cagcagtatggtagctcacctcggacg

SEQ ID NO: 48 - DNA, 27 bp, Artificial Sequence
  synthetic
atgcaaggtacacactggccgtggacg

SEQ ID NO: 49 - DNA, 27 bp, Artificial Sequence
  synthetic
atgcaaggttcacactggccgtacact

SEQ ID NO: 50 - DNA, 27 bp, Artificial Sequence
  synthetic
atgcaaggtacacactggccgctcact

SEQ ID NO: 51 - DNA, 27 bp, Artificial Sequence
  synthetic
caacagtatgataatctccctcccact

SEQ ID NO: 52 - DNA, 27 bp, Artificial Sequence
  synthetic
caacagtatgataatctcccattcact

SEQ ID NO: 53 - DNA, 27 bp, Artificial Sequence
  synthetic
caacagtatgataatctccccgtcact

SEQ ID NO: 54 - DNA, 27 bp, Artificial Sequence
  synthetic
caacagtatgataatctcccgatcacc

SEQ ID NO: 55 - DNA, 24 bp, Artificial Sequence
  synthetic
caacggatttacaatgccgacacc

SEQ ID NO: 56 - DNA, 30 bp, Artificial Sequence
  synthetic
caacagagttacagtacccccatgtacact

SEQ ID NO: 57 - DNA, 27 bp, Artificial Sequence
  synthetic
caacagagttacagtacccctctcact

SEQ ID NO: 58 - DNA, 27 bp, Artificial Sequence
  synthetic
caacagagttacagtactcctcccact